European Patent Specification EP 3 600 355 B1, published November 5, 2025. Title: Methods To Protect Transplanted Tissue From Rejection. Applicant: The Trustees of the University of Pennsylvania Riley, James L Ellis, Gavin. The sequence listing filed with the application follows.

SEQUENCE LISTING (48 sequences)

SEQ ID NO: 1 - protein, 245 aa, Artificial sequence
  HLA-A2 scFv
QVQLVQSGGGVVQPGGSLRVSCAASGVTLSDYGMHWVRQAPGKGLEWMAFIRNDGSDKYYADSVKGRFTISRDNSKKTVSLQMSSLRAEDTAVYYCAKNGESGPLDYWYFDLWGRGTLVTVSGGGGSGGGGSGGGGSDVVMTQSPSSLSASVGDRVTITCQASQDISNYLNWYQQKPGKAPKLLIYDASNLETGVPSRFSGSGSGTDFTFTISSLQPEDFATYYCQQYSSFPLTFGGGTKVDIKR

SEQ ID NO: 2 - DNA, 735 bp, Artificial sequence
  HLA-A2 scFv
caggtgcagctggtgcagtctgggggaggcgtggtccagcctggggggtccctgagagtctcctgtgcagcgtctggggtcaccctcagtgattatggcatgcattgggtccgccaggctccaggcaaggggctggagtggatggcttttatacggaatgatggaagtgataaatattatgcagactccgtgaagggccgattcaccatctccagagacaactccaagaaaacagtgtctctgcaaatgagcagtctcagagctgaagacacggctgtgtattactgtgcgaaaaatggcgaatctgggcctttggactactggtacttcgatctctggggccgtggcaccctggtcaccgtgtcgggtggcggtggctcgggcggtggtgggtcgggtggcggcggatctgatgttgtgatgactcagtctccatcctccctgtctgcatctgtaggagacagagtcaccatcacttgccaggcgagtcaggacattagcaactatttaaattggtatcagcagaaaccagggaaagcccctaagctcctgatctacgatgcatccaatttggaaacaggggtcccatcaaggttcagtggaagtggatctgggacagattttactttcaccatcagcagcctgcagcctgaggattttgcaacttattactgccaacaatatagtagttttccgctcactttcggcggagggaccaaagtggatatcaaacgt

SEQ ID NO: 3 - protein, 117 aa, Artificial sequence
  HLA-A2 scFv heavy chain (HC) variable region
QVQLVQSGGGVVQPGGSLRVSCAASGVTLSDYGMHWVRQAPGKGLEWMAFIRNDGSDKYYADSVKGRFTISRDNSKKTVSLQMSSLRAEDTAVYYCAKNGESGPLDYWYFDLWGRGT

SEQ ID NO: 4 - DNA, 351 bp, Artificial sequence
  HLA-A2 scFv heavy chain (HC) variable region
caggtgcagctggtgcagtctgggggaggcgtggtccagcctggggggtccctgagagtctcctgtgcagcgtctggggtcaccctcagtgattatggcatgcattgggtccgccaggctccaggcaaggggctggagtggatggcttttatacggaatgatggaagtgataaatattatgcagactccgtgaagggccgattcaccatctccagagacaactccaagaaaacagtgtctctgcaaatgagcagtctcagagctgaagacacggctgtgtattactgtgcgaaaaatggcgaatctgggcctttggactactggtacttcgatctctggggccgtggcacc

SEQ ID NO: 5 - protein, 5 aa, Artificial sequence
  HLA-A2 scFv HC CDR1
DYGMH

SEQ ID NO: 6 - protein, 17 aa, Artificial sequence
  HLA-A2 scFv HC CDR2
FIRNDGSDKYYADSVKG

SEQ ID NO: 7 - protein, 14 aa, Artificial sequence
  HLA-A2 scFv HC CDR3
NGESGPLDYWYFDL

SEQ ID NO: 8 - protein, 108 aa, Artificial sequence
  HLA-A2 scFv light chain (LC) variable region
DVVMTQSPSSLSASVGDRVTITCQASQDISNYLNWYQQKPGKAPKLLIYDASNLETGVPSRFSGSGSGTDFTFTISSLQPEDFATYYCQQYSSFPLTFGGGTKVDIKR

SEQ ID NO: 9 - DNA, 324 bp, Artificial sequence
  HLA-A2 scFv LC variable region
gatgttgtgatgactcagtctccatcctccctgtctgcatctgtaggagacagagtcaccatcacttgccaggcgagtcaggacattagcaactatttaaattggtatcagcagaaaccagggaaagcccctaagctcctgatctacgatgcatccaatttggaaacaggggtcccatcaaggttcagtggaagtggatctgggacagattttactttcaccatcagcagcctgcagcctgaggattttgcaacttattactgccaacaatatagtagttttccgctcactttcggcggagggaccaaagtggatatcaaacgt

SEQ ID NO: 10 - protein, 11 aa, Artificial sequence
  HLA-A2 scFv LC CDR1
QASQDISNYLN

SEQ ID NO: 11 - protein, 7 aa, Artificial sequence
  HLA-A2 scFv LC CDR2
DASNLET

SEQ ID NO: 12 - protein, 9 aa, Artificial sequence
  HLA-A2 scFv LC CDR3
QQYSSFPLT

SEQ ID NO: 13 - protein, 21 aa, Artificial sequence
  CD8 signal peptide
MALPVTALLLPLALLLHAARP

SEQ ID NO: 14 - DNA, 63 bp, Artificial sequence
  CD8 signal peptide
atggccttaccagtgaccgccttgctcctgccgctggccttgctgctccacgccgccaggccg

SEQ ID NO: 15 - protein, 45 aa, Artificial sequence
  CD8 hinge
TTTPAPRPPTPAPTIASQPLSLRPEACRPAAGGAVHTRGLDFACD

SEQ ID NO: 16 - DNA, 135 bp, Artificial sequence
  CD8 hinge
accacgacgccagcgccgcgaccaccaacaccggcgcccaccatcgcgtcgcagcccctgtccctgcgcccagaggcgtgccggccagcggcggggggcgcagtgcacacgagggggctggacttcgcctgtgat

SEQ ID NO: 17 - protein, 27 aa, Artificial sequence
  CD28 transmembrane domain
FWVLVVVGGVLACYSLLVTVAFIIFWV

SEQ ID NO: 18 - DNA, 81 bp, Artificial sequence
  CD28 transmembrane domain
ttttgggtgctggtggtggttggtggagtcctggcttgctatagcttgctagtaacagtggcctttattattttctgggtg

SEQ ID NO: 19 - protein, 41 aa, Artificial sequence
  CD28 intracellular domain
RSKRSRLLHSDYMNMTPRRPGPTRKHYQPYAPPRDFAAYRS

SEQ ID NO: 20 - DNA, 123 bp, Artificial sequence
  CD28 intracellular domain
aggagtaagaggagcaggctcctgcacagtgactacatgaacatgactccccgccgccccgggcccacccgcaagcattaccagccctatgccccaccacgcgacttcgcagcctatcgctcc

SEQ ID NO: 21 - protein, 112 aa, Artificial sequence
  CD3 zeta domain
RVKFSRSADAPAYQQGQNQLYNELNLGRREEYDVLDKRRGRDPEMGGKPRRKNPQEGLYNELQKDKMAEAYSEIGMKGERRRGKGHDGLYQGLSTATKDTYDALHMQALPPR

SEQ ID NO: 22 - DNA, 336 bp, Artificial sequence
  CD3 zeta domain
agagtgaagttcagcaggagcgcagacgcccccgcgtaccagcagggccagaaccagctctataacgagctcaatctaggacgaagagaggagtacgatgttttggacaagagacgtggccgggaccctgagatggggggaaagccgagaaggaagaaccctcaggaaggcctgtacaatgaactgcagaaagataagatggcggaggcctacagtgagattgggatgaaaggcgagcgccggaggggcaaggggcacgatggcctttaccagggtctcagtacagccaccaaggacacctacgacgcccttcacatgcaggccctgccccctcgc

SEQ ID NO: 23 - protein, 497 aa, Artificial sequence
  HLA-A2 CAR
MALPVTALLLPLALLLHAARPGSQVQLVQSGGGVVQPGGSLRVSCAASGVTLSDYGMHWVRQAPGKGLEWMAFIRNDGSDKYYADSVKGRFTISRDNSKKTVSLQMSSLRAEDTAVYYCAKNGESGPLDYWYFDLWGRGTLVTVSGGGGSGGGGSGGGGSDVVMTQSPSSLSASVGDRVTITCQASQDISNYLNWYQQKPGKAPKLLIYDASNLETGVPSRFSGSGSGTDFTFTISSLQPEDFATYYCQQYSSFPLTFGGGTKVDIKRSGTTTPAPRPPTPAPTIASQPLSLRPEACRPAAGGAVHTRGLDFACDFWVLVVVGGVLACYSLLVTVAFIIFWVRSKRSRLLHSDYMNMTPRRPGPTRKHYQPYAPPRDFAAYRSIDRVKFSRSADAPAYQQGQNQLYNELNLGRREEYDVLDKRRGRDPEMGGKPRRKNPQEGLYNELQKDKMAEAYSEIGMKGERRRGKGHDGLYQGLSTATKDTYDALHMQALPPR

SEQ ID NO: 24 - DNA, 1491 bp, Artificial sequence
  HLA-A2 CAR
atggccttaccagtgaccgccttgctcctgccgctggccttgctgctccacgccgccaggccgggatcccaggtgcagctggtgcagtctgggggaggcgtggtccagcctggggggtccctgagagtctcctgtgcagcgtctggggtcaccctcagtgattatggcatgcattgggtccgccaggctccaggcaaggggctggagtggatggcttttatacggaatgatggaagtgataaatattatgcagactccgtgaagggccgattcaccatctccagagacaactccaagaaaacagtgtctctgcaaatgagcagtctcagagctgaagacacggctgtgtattactgtgcgaaaaatggcgaatctgggcctttggactactggtacttcgatctctggggccgtggcaccctggtcaccgtgtcgggtggcggtggctcgggcggtggtgggtcgggtggcggcggatctgatgttgtgatgactcagtctccatcctccctgtctgcatctgtaggagacagagtcaccatcacttgccaggcgagtcaggacattagcaactatttaaattggtatcagcagaaaccagggaaagcccctaagctcctgatctacgatgcatccaatttggaaacaggggtcccatcaaggttcagtggaagtggatctgggacagattttactttcaccatcagcagcctgcagcctgaggattttgcaacttattactgccaacaatatagtagttttccgctcactttcggcggagggaccaaagtggatatcaaacgttccggaaccacgacgccagcgccgcgaccaccaacaccggcgcccaccatcgcgtcgcagcccctgtccctgcgcccagaggcgtgccggccagcggcggggggcgcagtgcacacgagggggctggacttcgcctgtgatttttgggtgctggtggtggttggtggagtcctggcttgctatagcttgctagtaacagtggcctttattattttctgggtgaggagtaagaggagcaggctcctgcacagtgactacatgaacatgactccccgccgccccgggcccacccgcaagcattaccagccctatgccccaccacgcgacttcgcagcctatcgctccatcgatagagtgaagttcagcaggagcgcagacgcccccgcgtaccagcagggccagaaccagctctataacgagctcaatctaggacgaagagaggagtacgatgttttggacaagagacgtggccgggaccctgagatggggggaaagccgagaaggaagaaccctcaggaaggcctgtacaatgaactgcagaaagataagatggcggaggcctacagtgagattgggatgaaaggcgagcgccggaggggcaaggggcacgatggcctttaccagggtctcagtacagccaccaaggacacctacgacgcccttcacatgcaggccctgccccctcgc

SEQ ID NO: 25 - protein, 5 aa, Artificial sequence
  linker
  REPEAT (1)..(5): Repeat n times. n is an integer of at least 1.
GSGGS

SEQ ID NO: 26 - protein, 4 aa, Artificial sequence
  linker
  REPEAT (1)..(4): Repeat n times. n is an integer of at least 1.
GGGS

SEQ ID NO: 27 - protein, 5 aa, Artificial sequence
  linker
  REPEAT (1)..(5): Repeat n times. n is an integer of at least 1.
GGGGS

SEQ ID NO: 28 - protein, 4 aa, Artificial sequence
  linker
GGSG

SEQ ID NO: 29 - protein, 5 aa, Artificial sequence
  linker
GGSGG

SEQ ID NO: 30 - protein, 5 aa, Artificial sequence
  linker
GSGSG

SEQ ID NO: 31 - protein, 5 aa, Artificial sequence
  linker
GSGGG

SEQ ID NO: 32 - protein, 5 aa, Artificial sequence
  linker
GGGSG

SEQ ID NO: 33 - protein, 5 aa, Artificial sequence
  linker
GSSSG

SEQ ID NO: 34 - protein, 5 aa, Artificial sequence
  linker
GGGGS

SEQ ID NO: 35 - protein, 15 aa, Artificial sequence
  linker
GGGGSGGGGSGGGGS

SEQ ID NO: 36 - DNA, 45 bp, Artificial sequence
  linker
ggtggcggtggctcgggcggtggtgggtcgggtggcggcggatct

SEQ ID NO: 37 - protein, 5 aa, Artificial sequence
  hinge
DKTHT

SEQ ID NO: 38 - protein, 4 aa, Artificial sequence
  hinge
CPPC

SEQ ID NO: 39 - protein, 15 aa, Artificial sequence
  hinge
CPEPKSCDTPPPCPR

SEQ ID NO: 40 - protein, 12 aa, Artificial sequence
  hinge
ELKTPLGDTTHT

SEQ ID NO: 41 - protein, 10 aa, Artificial sequence
  hinge
KSCDKTHTCP

SEQ ID NO: 42 - protein, 7 aa, Artificial sequence
  hinge
KCCVDCP

SEQ ID NO: 43 - protein, 7 aa, Artificial sequence
  hinge
KYGPPCP

SEQ ID NO: 44 - protein, 15 aa, Artificial sequence
  hinge
EPKSCDKTHTCPPCP

SEQ ID NO: 45 - protein, 12 aa, Artificial sequence
  hinge
ERKCCVECPPCP

SEQ ID NO: 46 - protein, 17 aa, Artificial sequence
  hinge
ELKTPLGDTTHTCPRCP

SEQ ID NO: 47 - protein, 12 aa, Artificial sequence
  hinge
SPNMVPHAHHAQ

SEQ ID NO: 48 - protein, 15 aa, Artificial sequence
  hinge
EPKSCDKTYTCPPCP